European Patent Application EP 4 166 663 A1, published April 19, 2023. Title: 目的タンパク質の製造方法  METHOD FOR PRODUCING A PROTEIN OF INTEREST. Applicant: ナガセケムテックス株式会社  Nagase ChemteX Corporation. The sequence listing filed with the application follows.

SEQUENCE LISTING (15 sequences)

SEQ ID NO: 1 - DNA, 1623 bp, Unknown
  phospholipase
atgctccgccaccggctccgccgtttacaccgtctgacccgcagtgcggcggtctcggccgtcgtcctggccgccctgcccgcggctccggccttcgcgagcagcccctcgcccgccccgcacctggacgccgtggagaaggcgctgcgcgaggtctcaccggggctggagggtgacgtctggcagcgcaccgacggcaacaagctggacgcctccgccgcggacccctccgactggctgctgcagacccccggttgctggggcgacgccgcgtgcaaggagcgtcccggcaccgagcgcctgctcgccaaggtgacggagaacatctccaaggccaggcgcacggtggacatctccacgctcgcgcccttcccgaacggtgcgttccaggacgcgatagccgccggcctcaaggcgtcggtcgcgtccggcaacaagccgaaggtccgcgtcctggtcggcgccgcgccggtctaccacatgaacgtactgccctcgaagtaccgggacgacctcaaggcccggctcggcaaggccgccgacgacatcacgctgaacgtcgcgtcgatgacgacgtcgaagaccagcttctcctggaaccactccaagctcctcgtcgtggacggcgagtcggccgtcaccggtggcatcaacagctggaaggacgactacgtcgacacccagcacccggtgaccgacgtggacctggcgctgaccggccccgccgcgagctccgccggccgctacctggacacgctctggacgtggacgtgccagaacaagagcaacatcgccagtgtgtggttcgcggcctcgggcggcgactgcatggccacgatggagaaggacgcgaaccccaggcccgccgggcccacgggcaacgtccccgtgatcgccgtgggcggcctcggcgtcggcatcaaggactccgaccccgcctggacgttccgcccgcagctgccctccgccccggacaccaagtgcgtcgtcggcctgcccgacaagaccaacgccgaccgtgactacgacacggtcaaccccgaggagagcgccctgcgggccctggtggccagcgccgaccgccagatcgtcatctcccagcaggacctgaacgccacctgcccgcccatcgcccgctacgacgtccgcctctacgacatcctcgccgccaagatggcggccggggtgaaggtgcgcatcgtcgtcagcgaccccgccaaccgcggcgcggtcggcagcggcggctactcgcaaatcaagtccctggccgagatcagcgacacgctccgcaaccgtctcgccctgctcaagggcggcgaccagcagaaggccaaggcggccatgtgctccaccctccagctggggaccttccgcagctccgcgagcgccacgtgggccgacgggcacccctacgccctgcaccacaagctggtggcggtcgacagctccgccttcaacatcggctccaagaacctctacccctcgtggctgcaggacttcggctacatcgtggagagcccggaggccgccaagcagcttgaggccaagctcctcgaccccgagtggaagttctcgcaggagaccgcgacggtcgaccacgcgcggggcgtctgctcgctctga

SEQ ID NO: 2 - DNA, 1197 bp, Unknown
  glucanase
atgctctcccgactcagacaccgtctgctcgccgtggccgcggccgcaggcctgaccggcgccctgctctcgttcggcgccgcaccgcccgcggacgccgcggtgcccgccaccatccccctgaagatcaccaacaactccgctcgtggcgacgccgtccacatctacaacctgggcacctcgctgacgaccggtcagcagggctgggcggacgagaacggaaccttccacgcctggcccgccggcggcaatccccccactcccgcaccggacgcgtccatccctggaccggccgcgggacagaccaagaccatccggatcccgaagctgtcgggacgcatctacttctcctacggccagaagctggacttccggctcaccaccggcggcctggtccagcccgccgtgcagaaccccagcgaccccaaccgcaacatcctcttcaactggtccgagtacacgctcaacgacggcgggctgtggctgaacagcacccaggtcgacatgttctccgcgccctacacggtcggcgtgcagcgcgccgacggcggcgtgaccagcgccggacagctcaaggccggtggctaccgcggggtgttcgacgcgctgcgggcccagccgggctggggcgggctgatccagacccggcccgacggcaccgtactgcgggcgctggcgccgctgtacggggtggagaccggggcgctgcccgcgtcggtcatggacgactacatcaaccgggtctggcagaagtacacgacgaccacgctcaccgtcacgcccttcggcgaccgtccggacaccaagtacttcggacgcgtctcgggcaacgtcatgaacttcaccaacacctccggcgcggtcgtcaccagcttccagaagccggacgcctccagcgtcttcggctgccaccggctcctggacgcgcccaacgaccaggtgcgcgggccgatctcgcgcacgctgtgcgccggcttcaaccgctcgacgctgctgagcaaccccaaccagcccgatccctcggcggcgaacttctaccgggacccggtgaccaaccactacgcccggatcatccacgagcgcatggccgacgggaaggcgtacgcgttcgccttcgacgacgtcggcaaccacgagtcgctggtgcacgacggcaacccggccgaggcgaggctcacgctcgccccgctcgactga

SEQ ID NO: 3 - DNA, 298 bp, Unknown
  metalloendopeptidase promoter
caggactgctcaggtgcgttttcgtatgcccgaacgcgcccggacgactccccgaacccgtccggtatttgagacgcgcccacagggcgccggggtgccacgaaacaaacccccgtcccagttcaccgcatagcggaaccaaacaaccgcactccggagaacgggagatcaaatccttgttgcgcccctgtcaatgacgcccaaacaatggcactctctcctcaattcgctcctgcaccacacctgcaccacagggcggtcgtacaaccggctgctccaacccccctcataggagaca

SEQ ID NO: 4 - DNA, 72 bp, Unknown
  phospholipase promoter
ggctcccgggagctgatagcttctccgcgttgatcttccgttcgcggaatcgttacttcgtttaaggatgca

SEQ ID NO: 5 - DNA, 206 bp, Unknown
  phospholipase terminator
gcatgcgacgactgagcgcccggacgttccggggcgcatgacgggggaatgcccgtaccgctgaggtacgggcattcccccgttcgctcatataactacgttcgaatatcggggaatgatccgatcgtcttcactccatagtgaacggatttcattccgtgtcgctccggatgcaaccatgcgctggccccgaaccgaccggaaat

SEQ ID NO: 6 - DNA, 30 bp, Artificial sequence
  sense primer
ctctcgccgtcggcgtgcagttgcttcctc

SEQ ID NO: 7 - DNA, 30 bp, Artificial Sequence
  antisense primer
catggacgccctccagggcacccggaagag

SEQ ID NO: 8 - DNA, 30 bp, Artificial Sequence
  sense primer
ggaattccaggactgctcaggtgcgttttc

SEQ ID NO: 9 - DNA, 30 bp, Artificial Sequence
  antisense primer
ggaattctcctggggtgtgacaccctacgc

SEQ ID NO: 10 - DNA, 34 bp, Artificial Sequence
  sense primer
ggtggggatatcggtcgtcctaccggctgctgtg

SEQ ID NO: 11 - DNA, 36 bp, Artificial Sequence
  antisense primer
ggtggggatatcgatcacccccgacagcggatcaag

SEQ ID NO: 12 - DNA, 31 bp, Artificial Sequence
  sense primer
ggttcggcgatatcagctcactcaaaggcgg

SEQ ID NO: 13 - DNA, 43 bp, Artificial Sequence
  antisense primer
ggaattcccggctcgcgatatcccgatttcggcctattggtta

SEQ ID NO: 14 - DNA, 30 bp, Artificial Sequence
  sense primer
ccatcgatcccccgacagcggatcaagggg

SEQ ID NO: 15 - DNA, 30 bp, Artificial Sequence
  antisense primer
ggcggtacctcgcgcccgactcgcctcgct